European Patent Application EP 4 226 948 A1, published August 16, 2023. Title: Oligonucleotide conjugate. Applicant: Sumitomo Dainippon Pharma Co., Ltd. The sequence listing filed with the application follows.

SEQUENCE LISTING (15 sequences)

SEQ ID NO: 1 - DNA, 26 bp, Artificial Sequence
  AS1411
ggtggtggtggttgtggtggtggtgg

SEQ ID NO: 2 - DNA, 26 bp, Artificial Sequence
  FAN-1524dI
  misc_feature (15)..(15): n is deoxyinosine
  misc_feature (24)..(24): n is deoxyinosine
ggtggtggtggttgnggtggtggngg

SEQ ID NO: 3 - RNA, 22 nt, Artificial Sequence
  EpCAM Aptamer
  modified_base (2)..(2): 2'-deoxy-2'-fluorocytidine
  modified_base (5)..(5): 2'-deoxy-2'-fluorocytidine
  modified_base (6)..(6): 2'-deoxy-2'-fluorouridine
  modified_base (9)..(10): 2'-deoxy-2'-fluorouridine
  modified_base (12)..(14): 2'-deoxy-2'-fluorocytidine
  modified_base (17)..(17): 2'-deoxy-2'-fluorouridine
  modified_base (18)..(18): 2'-deoxy-2'-fluorocytidine
  modified_base (20)..(22): 2'-deoxy-2'-fluorouridine
gcgacugguuacccggucguuu

SEQ ID NO: 4 - DNA, 38 bp, Artificial Sequence
  EpCAM Aptamer
  misc_feature (1)..(10): DNA fragment
  misc_feature (11)..(29): RNA fragment
  modified_base (12)..(12): 2'-deoxy-2'-fluorocytidine
  modified_base (14)..(14): 2'-deoxy-2'-fluorouridine
  modified_base (16)..(16): 2'-deoxy-2'-fluorouridine
  modified_base (17)..(19): 2'-deoxy-2'-fluorocytidine
  modified_base (20)..(23): 2'-deoxy-2'-fluorouridine
  modified_base (24)..(24): 2'-deoxy-2'-fluorocytidine
  modified_base (26)..(26): 2'-deoxy-2'-fluorocytidine
  modified_base (28)..(28): 2'-deoxy-2'-fluorouridine
  misc_feature (30)..(38): DNA fragment
cgcgcgccgcacguaucccuuuucgcguacggcgcgcg

SEQ ID NO: 5 - RNA, 79 nt, Artificial Sequence
  FB4
gggcgaauuccgcgugugcugagggcggaagaacuaauuugggacggauugcggccguugucuguggcguccguucggg

SEQ ID NO: 6 - DNA, 50 bp, Artificial Sequence
  GS24
gcgtgtgcacacggtcacttagtatcgctacgttctttggttccgttcgg

SEQ ID NO: 7 - DNA, 21 bp, Artificial Sequence
  Atp5b-siRNA sense strand
  modified_base (1)..(1): 2'-deoxy-2'-fluorouridine 5'-thiophosphate
  misc_feature (1)..(19): RNA fragment
  modified_base (2)..(2): 2'-O-methylguanosine 5'-thiophosphate
  modified_base (3)..(3): 2'-deoxy-2'-fluorouridine
  modified_base (4)..(4): cm
  modified_base (5)..(5): 2'-deoxy-2'-fluoroadenosine
  modified_base (6)..(6): um
  modified_base (7)..(7): 2'-deoxy-2'-fluorouridine
  modified_base (8)..(9): 2'-deoxy-2'-fluoroguanosine
  modified_base (10)..(10): 2'-O-methyladenosine
  modified_base (11)..(11): 2'-deoxy-2'-fluoroguanosine
  modified_base (12)..(12): 2'-O-methyladenosine
  modified_base (13)..(13): 2'-deoxy-2'-fluoroadenosine
  modified_base (14)..(14): cm
  modified_base (15)..(15): 2'-deoxy-2'-fluorocytidine
  modified_base (16)..(16): um
  modified_base (17)..(17): 2'-deoxy-2'-fluoroadenosine
  modified_base (18)..(18): um
  modified_base (19)..(19): 2'-deoxy-2'-fluorouridine
  misc_feature (20)..(21): DNA fragment
ugucauuggagaaccuauutt

SEQ ID NO: 8 - DNA, 21 bp, Artificial Sequence
  Atp5b-siRNA anti-sense strand
  modified_base (1)..(1): 2'-O-methyladenosine 3'-thiophosphate 5'-phosphate
  misc_feature (1)..(19): RNA fragment
  modified_base (2)..(2): 2'-deoxy-2'-fluoroadenosine 5'-thiophosphate
  modified_base (3)..(3): um
  modified_base (4)..(4): 2'-deoxy-2'-fluoroadenosine
  modified_base (5)..(5): gm
  modified_base (6)..(6): 2'-deoxy-2'-fluoroguanosine
  modified_base (7)..(7): um
  modified_base (8)..(8): 2'-deoxy-2'-fluorouridine
  modified_base (9)..(9): cm
  modified_base (10)..(10): 2'-deoxy-2'-fluorouridine
  modified_base (11)..(12): cm
  modified_base (13)..(13): 2'-O-methyladenosine
  modified_base (14)..(14): 2'-deoxy-2'-fluoroadenosine
  modified_base (15)..(15): um
  modified_base (16)..(16): 2'-deoxy-2'-fluoroguanosine
  modified_base (17)..(17): 2'-O-methyladenosine
  modified_base (18)..(18): 2'-deoxy-2'-fluorocytidine
  modified_base (19)..(19): 2'-O-methyladenosine 5'-thiophosphate
  misc_feature (20)..(21): DNA fragment
  modified_base (20)..(20): thymidine 5'-thiophosphate
aauagguucuccaaugacatt

SEQ ID NO: 9 - DNA, 21 bp, Artificial Sequence
  scramble-siRNA sense strand
  modified_base (1)..(1): 2'-deoxy-2'-fluoroguanosine 5'-thiophosphate
  misc_feature (1)..(19): RNA fragment
  modified_base (2)..(2): 2'-O-methylcytidine 5'-thiophosphate
  modified_base (3)..(3): 2'-deoxy-2'-fluorouridine
  modified_base (4)..(4): 2'-O-methyladenosine
  modified_base (5)..(5): 2'-deoxy-2'-fluoroguanosine
  modified_base (6)..(6): 2'-O-methyladenosine
  modified_base (7)..(7): 2'-deoxy-2'-fluorocytidine
  modified_base (8)..(8): 2'-deoxy-2'-fluorouridine
  modified_base (9)..(9): 2'-deoxy-2'-fluoroguanosine
  modified_base (10)..(10): um
  modified_base (11)..(11): 2'-deoxy-2'-fluorouridine
  modified_base (12)..(12): um
  modified_base (13)..(13): 2'-deoxy-2'-fluoroadenosine
  modified_base (14)..(14): 2'-O-methyladenosine
  modified_base (15)..(15): 2'-deoxy-2'-fluorocytidine
  modified_base (16)..(16): um
  modified_base (17)..(17): 2'-deoxy-2'-fluoroguanosine
  modified_base (18)..(18): 2'-O-methyladenosine
  modified_base (19)..(19): 2'-deoxy-2'-fluorouridine
  misc_feature (20)..(21): DNA fragment
gcuagacuguuuaacugautt

SEQ ID NO: 10 - DNA, 21 bp, Artificial Sequence
  scramble-siRNA anti-sense strand
  modified_base (1)..(1): 2'-O-methyladenosine 3'-thiophosphate 5'-phosphate
  misc_feature (1)..(19): RNA fragment
  modified_base (2)..(2): 2'-deoxy-2'-fluorouridine 5'-thiophosphate
  modified_base (3)..(3): cm
  modified_base (4)..(4): 2'-deoxy-2'-fluoroadenosine
  modified_base (5)..(5): gm
  modified_base (6)..(6): 2'-deoxy-2'-fluorouridine
  modified_base (7)..(7): um
  modified_base (8)..(8): 2'-deoxy-2'-fluoroadenosine
  modified_base (9)..(9): 2'-O-methyladenosine
  modified_base (10)..(10): 2'-deoxy-2'-fluoroadenosine
  modified_base (11)..(11): cm
  modified_base (12)..(12): 2'-O-methyladenosine
  modified_base (13)..(13): gm
  modified_base (14)..(14): 2'-deoxy-2'-fluorouridine
  modified_base (15)..(15): cm
  modified_base (16)..(16): 2'-deoxy-2'-fluorouridine
  modified_base (17)..(17): 2'-O-methyladenosine
  modified_base (18)..(18): 2'-deoxy-2'-fluoroguanosine
  modified_base (19)..(19): 2'-O-methylcytidine 5'-thiophosphate
  misc_feature (20)..(21): DNA fragment
  modified_base (20)..(20): thymidine 5'-thiophosphate
aucaguuaaacagucuagctt

SEQ ID NO: 11 - DNA, 16 bp, Artificial Sequence
  Malat1-ASO
  misc_feature (1)..(3): RNA fragment
  misc_feature (1)..(15): phosphorothioate modified nucleotides
  modified_base (1)..(1): 2'-O,4'-C-methylene-5-methylcytidine bridged 5'-thiophosphate
  modified_base (2)..(2): 2'-O,4'-C-methylenethymidine bridged 5'-thiophosphate
  modified_base (3)..(3): 2'-O,4'-C-methyleneadenosine bridged 5'-thiophosphate
  misc_feature (4)..(13): DNA fragment
  misc_feature (14)..(16): RNA fragment
  modified_base (14)..(14): 2'-O,4'-C-methylenethymidine bridged 5'-thiophosphate
  modified_base (15)..(15): 2'-O,4'-C-methyleneguanosine bridged 5'-thiophosphate
  modified_base (16)..(16): 2'-O,4'-C-methylene-5-methylcytidine bridged 5'-phosphate
ctagttcactgaatgc

SEQ ID NO: 12 - DNA, 22 bp, Artificial Sequence
  ATP5B-forward primer
ggtcctgagactttgggcagaa

SEQ ID NO: 13 - DNA, 20 bp, Artificial Sequence
  ATP5B-reverse primer
cctcagcatgaatgggagca

SEQ ID NO: 14 - DNA, 20 bp, Artificial Sequence
  GAPDH-forward primer
gcaccgtcaaggctgagaac

SEQ ID NO: 15 - DNA, 19 bp, Artificial Sequence
  GAPDH-reverse primer
tggtgaagacgccagtgga